European Patent Specification EP 3 502 243 B1, published October 9, 2024. Title: Variants of fungal cellulase. Applicant: AB Enzymes Oy. The sequence listing filed with the application follows.

SEQUENCE LISTING (3 sequences)

SEQ ID NO: 1 - protein, 235 aa, Melanocarpus albomyces
MRSTPVLRALLAAALPLGALAANGQSTRYWDCCKPSCGWAGKGPVNQPVYSCDANFQRIHDFDAVSGCEGGPAFSCADHSPWAINDNLSYGFAATALSGQTEESWCCACYALTFTSGPVAGKTMVVQSTSTGGDLGSNHFDLNIPGGGVGLFDGCTPQFGGLPGARYGGISSRQECDSFPEPLKPGCQWRFDWFQNADNPSFTFERVQCPEELVARTGCRRHDDGGFAVFKAPSA

SEQ ID NO: 2 - DNA, 849 bp, Melanocarpus albomyces
atgcgctctactcccgttctccgcgccctcctggccgcagcattgcccctcggggccctcgccgccaacggtcagtccacgaggtaactgatcacccgcctcattacgcgtgccgaccggaccgcgttcagggctcactgctcaccgcatccagatactgggactgctgcaagccgtcgtgcggctgggccggaaagggccccgtgaaccagcccgtctactcgtgcgacgccaacttccagcgcatccacgacttcgatgccgtctcgggctgcgagggcggccccgccttctcgtgcgccgaccacagcccctgggccattaatgacaacctctcgtacggcttcgcggcgactgcactcagcggccagaccgaggagtcgtggtgctgtgcctgctacgcgtgagtgtgcttgggcccaacgtcggtgattccggagttcagaccactgacccagcgacccgctcgccagtctgacctttacatcgggtcccgtggccggcaagaccatggtcgtccagtcgaccagcacgggcggcgacctcggcagcaaccacttcgacctcaacatccccggcggcggcgtcggcctcttcgacggctgcactccccagttcggcggcctcccgggcgcacggtacggcggcatctcgtcgcgccaggagtgcgactcgttccccgagccgctcaagcccggctgccagtggcgcttcgactggttccagaacgccgacaacccgtcctttaccttcgagcgggtccagtgccccgaggagctggtcgctcggaccggctgcaggcgccacgacgacggcggcttcgccgtcttcaaggcccccagcgcctga

SEQ ID NO: 3 - protein, 214 aa, Melanocarpus albomyces
ANGQSTRYWDCCKPSCGWAGKGPVNQPVYSCDANFQRIHDFDAVSGCEGGPAFSCADHSPWAINDNLSYGFAATALSGQTEESWCCACYALTFTSGPVAGKTMVVQSTSTGGDLGSNHFDLNIPGGGVGLFDGCTPQFGGLPGARYGGISSRQECDSFPEPLKPGCQWRFDWFQNADNPSFTFERVQCPEELVARTGCRRHDDGGFAVFKAPSA